European Patent Specification EP 3 762 403 B1, published May 1, 2024. Title: A neurotrophic peptide for the therapeutic treatment of neurodegenerative and/or inflammatory diseases. Applicant: Consiglio Nazionale delle Ricerche. The sequence listing filed with the application follows.

SEQUENCE LISTING (9 sequences)

SEQ ID NO: 1 - protein, 296 aa, Homo sapiens
MASSNGHFNEVLASGRAVQGAGWHAGPKLSSASGPNNSFTKGAAFYPGHTEVHSVMSMLFYTLITAFLIGIQAEPHSESNVPAGHTIPQAHWTKLQHSLDTALRRARSAPAAAIAARVAGQTRNITVDPRLFKKRRLRSPRVLFSTQPPREAADTQDLDFEVGGAAPFNRTHRSKRSSSHPIFHRGEFSVCDSVSVWVGDKTTATDIKGKEVMVLGEVNINNSVFKQYFFETKCRDPNPVDSGCRGIDSKHWNSYCTTTHTFVKALTMDGKQAAWRFIRIDTACVCVLSRKAVRRA

SEQ ID NO: 2 - DNA, 1159 bp, Homo sapiens
ggaaatgtcactgcagaagagcaagggagctcaagacgcgatggcagctgtcactccagagtggtgtggagtgggacggtatctgatgtgtcctcagattcggtttcccttgggatgtgtttggtgctgactgcttgtgatccatgttttcttggatgcaggttggtagaggtgcagcaatttttgcagtgaaactgaagtccagctgctcaaacagaaatggcctcatctaatggacactttaatgaagttttggccagtggtcgtgcagtccaaggggctggatggcatgctggacccaagctcagctcagcgtccggacccaataacagttttaccaagggagcagctttctatcctggccacactgaggtgcatagcgtaatgtccatgttgttctacactctgatcacagcttttctgatcggcatacaggcggaaccacactcagagagcaatgtccctgcaggacacaccatcccccaagcccactggactaaacttcagcattcccttgacactgcccttcgcagagcccgcagcgccccggcagcggcgatagctgcacgcgtggcggggcagacccgcaacattactgtggaccccaggctgtttaaaaagcggcgactccgttcaccccgtgtgctgtttagcacccagcctccccgtgaagctgcagacactcaggatctggacttcgaggtcggtggtgctgcccccttcaacaggactcacaggagcaagcggtcatcatcccatcccatcttccacaggggcgaattctcggtgtgtgacagtgtcagcgtgtgggttggggataagaccaccgccacagacatcaagggcaaggaggtgatggtgttgggagaggtgaacattaacaacagtgtattcaaacagtacttttttgagaccaagtgccgggacccaaatcccgttgacagcgggtgccggggcattgactcaaagcactggaactcatattgtaccacgactcacacctttgtcaaggcgctgaccatggatggcaagcaggctgcctggcggtttatccggatagatacggcctgtgtgtgtgtgctcagcaggaaggctgtgagaagagcctgacctgccgacacgctccctccccctgccccttctacactctcctgggccc

SEQ ID NO: 3 - DNA, 891 bp, Homo sapiens
atggcctcatctaatggacactttaatgaagttttggccagtggtcgtgcagtccaagggcgtggatggcatgctggacccaagctcagctcagcgtccggacccaataacagttttaccaagggagcagctttctatcctggccacactgaggtgcatagcgtaatgtccatgttgttctacactctgatcacagcttttctgatcggcatacaggcggaaccacactcagagagcaatgtccctgcaggacacaccatcccccaagcccactggactaaacttcagcattcccttgacactgcccttcgcagagcccgcagcgccccggcagcggcgatagctgcacgcgtggcggggcagacccgcaacattactgtggaccccaggctgtttaaaaagcggcgactccgttcaccccgtgtgctgtttagcacccagcctccccgtgaagctgcagacactcaggatctggacttcgaggtcggtggtgctgcccccttcaacaggactcacaggagcaagcggtcatcatcccatcccatcttccacaggggcgaattctcggtgtgtgacagtgtcagcgtgtgggttggggataagaccaccgccacagacatcaagggcaaggaggtgatggtgttgggagaggtgaacattaacaacagtgtattcaaacagtacttttttgagaccaagtgccgggacccaaatcccgttgacagcgggtgccggggcattgactcaaagcactggaactcatattgtaccacgactcacacctttgtcaaggcgctgaccatggatggcaagcaggctgcctggcggtttatccggatagatacggcctgtgtgtgtgtgctcagcaggaaggctgtgagaagagcctga

SEQ ID NO: 4 - DNA, 21 bp, Homo sapiens
tggcctcatctaatggacact

SEQ ID NO: 5 - DNA, 20 bp, Homo sapiens
gaaagctgctcccttggtaa

SEQ ID NO: 6 - DNA, 20 bp, Homo sapiens
agagagcgctgggagccgga

SEQ ID NO: 7 - DNA, 21 bp, Homo sapiens
ggacgctgagctgagcttggg

SEQ ID NO: 8 - DNA, 20 bp, Homo sapiens
atggcctcatctaatggaca

SEQ ID NO: 9 - DNA, 18 bp, Homo sapiens
ggctcttctcacagcctt